European Patent Specification EP 3 775 223 B1, published July 9, 2025. Title: Method for increasing the expression level of a nucleic acid molecule of interest in a cell. Applicant: KWS SAAT SE. The sequence listing filed with the application follows.

SEQUENCE LISTING (56 sequences)

SEQ ID NO: 1 - DNA, 57 bp, Zea mays
aacccggacccggtaggaaggagctataaagacaagccaaacgagggcatcccttct

SEQ ID NO: 2 - DNA, 57 bp, Zea mays
cgctataaaatatccccacgctgcttcgccctgcccaccacagcatccgcagttccc

SEQ ID NO: 3 - DNA, 57 bp, Zea mays
tgctgttagcggtataaaaagcggaaaccctagcattcgccgcgagcttatcactta

SEQ ID NO: 4 - DNA, 60 bp, Zea mays
gggactcggcgacaggccttttgtagaccgcagccggcaccatctcttgccgcacccccc

SEQ ID NO: 5 - DNA, 60 bp, Zea mays
cccctcttaaaagccgcctctcgccgccgcccgcaaaccctcatttttctctctcctgcg

SEQ ID NO: 6 - DNA, 60 bp, Zea mays
ccaccataaatgcgccgcggccgtcctcgctgcccaacccttgctcgctgcgccgccgcc

SEQ ID NO: 7 - DNA, 60 bp, Zea mays
ggcgttaatatctcccctcccttccctcttctggtctccgccccgctccttgcctccgat

SEQ ID NO: 8 - DNA, 60 bp, Zea mays
cgttttttttacgctgtcaatgcataacctgcgttggcattccgcctgctggacttcctc

SEQ ID NO: 9 - DNA, 60 bp, Zea mays
cgcccgccgtcataaatagccagccccatccccagcttctttccccaacctcatcttctc

SEQ ID NO: 10 - DNA, 60 bp, Zea mays
cgcccgccgtaataaatagacaccccctccacaccctctttccccaacctcgtgttgttc

SEQ ID NO: 11 - DNA, 60 bp, Zea mays
tgctgctagcagtataaatatgctgaaagcctgaaaccctaggcgaagcttatcgcttat

SEQ ID NO: 12 - DNA, 60 bp, Zea mays
gtcggctttaaaaggacacgagcgcttaaacccccaccccatatccgcatccgctgcctc

SEQ ID NO: 13 - DNA, 60 bp, Zea mays
gccggctttaaaaacgcacacaagcgctaaaaccctctccaccgtccacctcagctccca

SEQ ID NO: 14 - DNA, 60 bp, Zea mays
cccgactacatcaaccaacgcgtatcggcggtggcaaaccctctagcttcccactccgct

SEQ ID NO: 15 - DNA, 20 bp, Zea mays
tataaagacaagccaaacga

SEQ ID NO: 16 - DNA, 20 bp, Zea mays
gctataaaatatccccacgc

SEQ ID NO: 17 - DNA, 20 bp, Zea mays
gtataaaaagcggaaaccct

SEQ ID NO: 18 - DNA, 20 bp, Zea mays
gctataaagacaagccaaac

SEQ ID NO: 19 - DNA, 20 bp, Artificial Sequence
  fusion of two contiguous streches of E53
gctataaagagcatcccttc

SEQ ID NO: 20 - DNA, 60 bp, Beta vulgaris
atgtaaaaaaaaagcttatataaagggaatcagacatgaggttttggcataaaaactatc

SEQ ID NO: 21 - DNA, 60 bp, Beta vulgaris
ccccctcacccctacatatacaccactctctccttcaatcttcttcatcactctcatttt

SEQ ID NO: 22 - DNA, 60 bp, Beta vulgaris
gcgtaattatgaacgttatataaaccggttacaattacaacctatcacaccaaaaagcaa

SEQ ID NO: 23 - DNA, 60 bp, Beta vulgaris
ccacctccttcaaacctatttatactccctcacctccttcactacctcctcgcttcaccc

SEQ ID NO: 24 - DNA, 60 bp, Beta vulgaris
tctacacttcctttagtatatttagcctcaaattactactggtcacttatacatttctca

SEQ ID NO: 25 - DNA, 60 bp, Beta vulgaris
gtcggtcaaacaagtctttaaatacagcctattcccttcattggtttctcatccttcatt

SEQ ID NO: 26 - DNA, 60 bp, Beta vulgaris
accctaaaacactccttatataattcactccctcacatttcaatttccgcctcctatact

SEQ ID NO: 27 - DNA, 60 bp, Beta vulgaris
gtttctctctctctcctttaaataaaaccctaactttcttcaccactctcactcacactc

SEQ ID NO: 28 - DNA, 60 bp, Beta vulgaris
cttcctctcctcaacataataaaggatagcaagtcacacattcaatcgcctctctctcct

SEQ ID NO: 29 - DNA, 60 bp, Beta vulgaris
gatactccatttccattatttaaggagtgcaagtgtgggtgtatgaaagtaaggtaccaa

SEQ ID NO: 30 - DNA, 60 bp, Beta vulgaris
ttcctcatttctccagtataagaaccaccaccacccttgttctcccacaaacgcaaaatc

SEQ ID NO: 31 - DNA, 1754 bp, Zea mays
atcggacccaaatcatagacacatgatgatataataacagacaaccaaaattgagagtggcaaaatagcaaatttctgatagtcatgtgatagagaatagtagacaattttgacataatatatgtacactaattagtcaacaaaagcgatattgcggttaaaacagtgattgccagtgttttgacccgagtgtcctaaccaaccaataaagtaaatttatgctatgtgtcctcgtccagatggatgatgcaagaagacacaagatttattttggttcggacaatagaaggcctactttcagcggagggggatgggatttatattatcttgcacctaagtgcttgtagtagaaggtacaagttagtcgagagagagagagaatcccaactctctgcggatgattgaggcaagtgtcaatatcggccgcggagggcaataggtgaagtgtattgtcctcctcccttgcaagccttggactccttttatagccttaatgagggaatcaaggagtaataattagttgaagactgattaagaaacagtccatctgttagtttttttgtttaaataggctaaagctaattttatctagttcttaattagctaataattattatttcgtaggatccaaaccattcctaagctatagtgctattatatcaagtgtagatctatatgtactcaaggtcatgatgtttgcaaaccaacaatgaaatttatcgcacacattggtcatggcagatcaacttttttgccacaaaacaaacaagaatagtgcaaacgaagttgcataaaatgaaacaatatattatgtgaatagttgcatggtttatcttgctagttccattttaacacacacacatatcttgctagttccattttaacttctacttgcacaattccaaaaggaacctaaatttcatttaccgatgagtcacaagaaacttagatctaattaaatttaaagaaaaatagcaatatttatatttttaaatatatttattataaaaatttatctcatattctagctaatgatatttattatgcatcataactattaaatatatagctatatatatatatatttcataagtttcatgttgtttaacttaatagagatttatatttttagggctagtttggcaaactatttttccaaaggattttcatttctataaagaaaattatttttttaaaaaaaatagaaatctcttgaaagaatagaattgttaaactactcttagacaaataaagagtatccttggttcgtggctaaccgtatcatattttatctaagttagttgttccaattaaagaactaattttatacacaaaagttaagtaaagtatagcaaattagtccgcgaaccaaatatgaccgaaatatcgaggagtgaggaggcttaacccttcccatgtgtgtatctactgttacaccgtgagctacaaagttactggcacaaacgtatagaggatggtgaggacatgggaagataaaatcctggtccagcaagatccgttcttccaaatgggatcaggtgattggctccagttcctcctcccctcagcaccaccagtctcctccagtccagctcccgtcttctccgcctcaagagtctcagaccaacggcaaagttctagaagcacggttgcacgggcagcacggcataacacctccctccactgatccagttccagtcgcccaacgccccaacgtcttctcttgcaaatcgcaagcaaacttcctgttcacg

SEQ ID NO: 32 - DNA, 658 bp, Zea mays
gttggctacttgagttagattttggttgtgtttcatccccacgtacgtccagcaaagaaaaattgaagctagtgcatgcatggttcgtcatcaaatgcatggccggccggatacaaatttgaactgtagctatcgacgtacgcatgtattaatttatatcagagaagacaaggaacacagatacatacatgtcgaaacaatcattttctatggcacttgagctagctagcatacaattttgttttaaatgaaatgaaactgaagacgatcgatcgaattgaaggttgtggttcgtgagcaatgcaatgcagtttcacagaacgttgccaatgcaacaagccaccaagaaaagagaagtctactcgatcttgcaatgattaggcttggatgatgcgtggggccacgtacgtatggacatcgaagaaccccatcctcagcgtgtggcctgagggtgatggcaaagctgatccacacattgcggccccctttcccccctcagagaccctgacctcccgagcacagccagccaccgcgcaacgccggccaccaccaccaccaccatacctgctagcgctagctctctttatttaacgccgccgtgtgcgtgcctcgacgacctcactactttgagctgcaaggtccgaactaaaaagcaccg

SEQ ID NO: 33 - DNA, 1700 bp, Beta vulgaris
tataagttcaaacttcaatacaggtattttcgggatgtgattaccttacaatttctcattttcaaagaattttacctgtgcagctatgttggataacctgtgcgagattccgtttcagtaggacactttttttttttaccaataaaaaaaaacttataagttcatgagctaatttttatagatagtttaaagtaccgggtggaggatgaatagttgagttttttcttcaaaattagatacttcctccgttttttattagatgttacacttttcaaatcacggactcctaggtaatttttggagaggagagagatagagagaatgaaaaacaaaagggtcccatgtgagtatgtgataggagagagatagagagaatttattacccaaaataaaagtgtaacatctaattcaaaacttcctaaaatagaaagtgtaacatctaaaaaaaacggaggaagtatttgaatttgatatagatattgtgtctttgtgtgtgttgaatttcaattcccagttccctaaaaaaaatttacaattgcaatttcgagattatgatgtaaattaaatttgagagactagaaagtatttggtcaacccaaaaaaaaaatatcaatacttatataaatcaaaaacataatagagaatccaattttactaaaaatattagtaattttgattaaaataatctattaaaatgaactctaaccttcacataatttccacatattattaatcaacaaaataagcatcacaaattattagaataggcgatctaattttaacataaaattagacgaattcaaattgaatttttctaacaagctcattccatttcacgcaacccaaaattatcctagtcagtagtcatccattcttttctcattcctttattcttgattatcgaactacaacagataatttcaaaaaaaaactaaattggtagtcttaactgattaaactacttactaaatggattaaagaatgtcattactgaatagattaaactgattacgaaatagattaacttggtccctaaatagattaaattagttactatattaaaattaggcgatctcttacaaaaccaactgaataagcatagctctgtatattacctagatttcaactaaatcaaaaccccttacagttcaatctagagctgatcattttggctcggcccgtcccatttttgggccgggttttagtcagatttttttggcccgcggtcgggcccggcccgatttttttggctttgggcaagccaaaaacgacttttcagtttattttttggcccgacccgtttttacccgcaaaagcccgctaatttaggtccgcactttgggcacaaaaatttagcccgaacttaaacctggcccgacccatgatcacctctagtttaatccaaactaaaaaactacacaagttagccaaaaattatgtctactttgtacaactttataaaatacacacagtagttgatatcttgatgattaactccttttgaagtttgactacacaccaaccccaaacacacccactttttcccccctcttgtcaccaaccccccctcctctttagccaccaaagtttggttggtgagtcctccataactgctaaattctctcttttttctctctcctaaaaaactaaaacccaccaaaatttcagacatcaaaaaaattacaagtgaaggaaacaat

SEQ ID NO: 34 - DNA, 991 bp, Beta vulgaris
aaagaaggaaaggaaggaatttgaacatgtgacctatcgttcacagcacctcaatcttaatcactagaccaaaacatccttggttcttgcgcaagaaggttggctagaaattttttgtaaaaacactagccccgctcagttcataatgagaatgtcgatgtcaccaaagggatattaaatgaatggaattgggatatggatggaatataatgaaatagagccactttgaggttccctatgaaatgaggcatggaagggagccactacgaaaaagttccgggagttacgaaggaagcttcgagctcatattggtcatgaacccgattactgagtctaataagttcaattgaaaagaaaaagtcttatgttctaaaagaacttttcgtgcggtttgcatgagttcatagtccatataatataatgcaggaatgaagttctcagttgattcttccacacccgtccctcaccccctaggccccaccttcaccccgccgaaaaaaataaagaaaatccaacgttatttttcttagaaatgacagtttgatatagaaaggaaaaataataataaaaaaaaaaagtgttggcgttttcattttcaacctcagtatgttggtttgccccaacaagttctgaaccaattggcgatgtaatcttataagaagaatctaacgttggtccattttgcttctacagttttgaaagttaggtgggccccattattatgttgatcctagaataattaattttggtaggctgagaagaggaaaaataaagaacaatgctaaaaacaagtgaaaaatatagttgcaactcatgatgcaacatgagatgcgatgaaatatgatagtaacttgagctcacaactctgtatataagtgctcatttggacacttattttctacaatttcctagtaactcagcttagcttcattcccgacttttttataaaagtcaggacgatcaatatctatctatttatctgtctgtctgt

SEQ ID NO: 35 - DNA, 35 bp, Zea mays
  misc_feature (10)..(32): n is a, c, g, or t
ttattattannnnnnnnnnnnnnnnnnnnnnntga

SEQ ID NO: 36 - DNA, 35 bp, Artificial Sequence
  Zm-prom1v3
  misc_feature (10)..(32): n is a, c, g, or t
gtataaaagnnnnnnnnnnnnnnnnnnnnnnntga

SEQ ID NO: 37 - DNA, 38 bp, Zea mays
aagataaaatcctggtccagcaagatccgttcttccaa

SEQ ID NO: 38 - DNA, 40 bp, Artificial Sequence
  ZmZEP1v1
aagtataaaagtcctggtccagcaagatccgttcttccaa

SEQ ID NO: 39 - DNA, 39 bp, Artificial Sequence
  ZmZEP1v2
aagctataaagagcatcccttcaagatccgttcttccaa

SEQ ID NO: 40 - DNA, 39 bp, Artificial Sequence
  ZmZEP1v3
aagctataaaatatccccacgcaagatccgttcttccaa

SEQ ID NO: 41 - DNA, 10 bp, Arabidopsis thaliana
tttcttcttc

SEQ ID NO: 42 - DNA, 15 bp, Zea mays
ctataaagacaagcc

SEQ ID NO: 43 - DNA, 15 bp, Zea mays
ctataaaatatcccc

SEQ ID NO: 44 - DNA, 15 bp, Zea mays
gtataaaaagcggaa

SEQ ID NO: 45 - DNA, 15 bp, Zea mays
tcttaaaagccgcct

SEQ ID NO: 46 - DNA, 15 bp, Zea mays
ccataaatgcgccgc

SEQ ID NO: 47 - DNA, 15 bp, Zea mays
tcataaatagccagc

SEQ ID NO: 48 - DNA, 15 bp, Zea mays
taataaatagacacc

SEQ ID NO: 49 - DNA, 15 bp, Zea mays
gtataaatatgctga

SEQ ID NO: 50 - DNA, 15 bp, Zea mays
ctttaaaaggacacg

SEQ ID NO: 51 - DNA, 15 bp, Zea mays
ctttaaaaacgcaca

SEQ ID NO: 52 - DNA, 687 bp, Zea mays
agaaacatagcattgtaaagtatatttgaagctctccaatatggttaaaattgaaaaaaaaaattgcacaactaggcgtatccagtgagaaaaggccttgccactctacgtatctgatgttgttaataatttcagaagtcgtcgtatataccatggggtgtttaattgtcgtatatacgatgggatgcttaattgtcgtatatacgatggtatgatgaaacaactgacttaaacatcacactgaacaatttcagaaaacgatccatgccgtcgtatatatacgacaacaaaataccagaagcaaacctcccagacccaaggggaaataaacgggcctgcttctggtcgctagcttgggggcgctggagctgcagtgcgtaggcccgtccgatccgtggctcgtctcggcatggccacacaaaccacgaacggtcgtcgtgcaccgcagcgcggcccccccgttctatcttctccagctccaaatggcgccatcgcggcggccgggttatcttgtccagacgtgcatcatatcctccgtgtgatccattcatccccgcgccgtgctagcttgctagttgcaagcaccagccgaccaccaaacggtagcgcacgcggacaatttaacagcatcaggtttaggccctgctgccgtcgtcgagcgcccgggccaccgcacacctgaaagca

SEQ ID NO: 53 - DNA, 24 bp, Zea mays
cagctccaaatggcgccatcgcgg

SEQ ID NO: 54 - DNA, 24 bp, Artificial Sequence
  modified target region in ZmSBPase promoter sequence, ZmSBPase_v1
cagctttaaatggcgccatcgcgg

SEQ ID NO: 55 - DNA, 24 bp, Artificial Sequence
  modified target region of ZmSBPase promoter sequence, ZmSBPase_v4
cagctctaaatggcgccatcgcgg

SEQ ID NO: 56 - DNA, 24 bp, Artificial Sequence
  modified target region of ZmSBPase promoter sequence, ZmSBPase_v5
cagcttcaaatggcgccatcgcgg